European Patent Specification EP 4 074 822 B1, published October 22, 2025. Title: Tagatose production composition and tagatose manufacturing method using the same. Applicant: CJ CheilJedang Corporation Korea Advanced Institute of Science and Technology. The sequence listing filed with the application follows.

SEQUENCE LISTING (13 sequences)

SEQ ID NO: 1 - DNA, 1308 bp, Unknown
  Kosmotoga olearia fructose-4-epimerase Wild type_ polynucleotide
atgaaaaaacatcctcttcaggacattgtttcattgcaaaaacagggaatacccaaaggggttttctctgtatgtagtgccaatagatttgttattgaaaccactctggaatatgcgaagatgaaagggacaacggttcttatagaggccacctgcaatcaggtaaaccagttcggtggctacaccggtatgactcctgctgatttcagagaaatggttttttctatcgctgaggatattggacttcccaaaaataaaatcatccttggtggcgaccatcttggcccaaatccctggaagggtcagccgtcagatcaggctatgcgtaacgccattgaaatgattcgagaatacgctaaagctgggtttaccaagcttcatctggatgccagcatgcgtcttgcagacgatccggggaacgaaaacgagccgctgaacccggaagttatagcggaaagaacagctcttctctgtcttgaagccgagagggcttttaaagaatccgccggttctctccggcctgtttacgttattggtacggatgttccgccaccgggtggagcgcaaaacgaaggtaaatcgattcatgtaaccagtgttcaggattttgagcgtaccgttgagttgaccaaaaaggcatttttcgaccatggtttgtatgaagcctggggaagggtgattgcggttgttgtgcaaccgggagtagaattcgggaatgaacatatattcgaatatgatagaaatcgagcgagagaacttactgaggcgataaaaaagcatccaaatatagtttttgaaggtcactcgacagattatcaaacggcaaaagcattgaaagaaatggtagaagacggtgtagccatactcaaggttgggccagctctaacatttgcgctcagagaggctttttttgcgttgagcagcattgaaaaagagttattttatgatacacccgggctttgttcaaactttgttgaagttgtcgagagagcgatgcttgacaatccaaaacattgggaaaaatattaccagggagaagagagagaaaatagattagcccgtaaatacagctttctcgatcgcttgaggtattactggaatcttcctgaggttagaacagcggtgaataagctgataaccaaccttgaaacaaaagaaatcccgttaacgcttataagccagttcatgccgatgcagtaccaaaaaatcagaaacggtttgctaagaaaggatccaataagccttataaaagatcgaattacccttgttcttgatgactactatttcgcaactcaccctgaatgttga

SEQ ID NO: 2 - protein, 435 aa, Unknown
  Kosmotoga olearia fructose-4-epimerase_amino acid
MKKHPLQDIVSLQKQGIPKGVFSVCSANRFVIETTLEYAKMKGTTVLIEATCNQVNQFGGYTGMTPADFREMVFSIAEDIGLPKNKIILGGDHLGPNPWKGQPSDQAMRNAIEMIREYAKAGFTKLHLDASMRLADDPGNENEPLNPEVIAERTALLCLEAERAFKESAGSLRPVYVIGTDVPPPGGAQNEGKSIHVTSVQDFERTVELTKKAFFDHGLYEAWGRVIAVVVQPGVEFGNEHIFEYDRNRARELTEAIKKHPNIVFEGHSTDYQTAKALKEMVEDGVAILKVGPALTFALREAFFALSSIEKELFYDTPGLCSNFVEVVERAMLDNPKHWEKYYQGEERENRLARKYSFLDRLRYYWNLPEVRTAVNKLITNLETKEIPLTLISQFMPMQYQKIRNGLLRKDPISLIKDRITLVLDDYYFATHPEC

SEQ ID NO: 3 - DNA, 1305 bp, Artificial Sequence
  Kosmotoga olearia fructose-4-epimerase Variant polynucleotide_ polynucleotide
atgaaaaagcatccattgcaggacatcgtatcactgcagaagcagggtatccccaagggcgtcttctcagtctgttccgctaaccgtttcgtcatcgagaccactctggaatacgccaagatgaagggcactacggttcttattgaagcaacctgtaaccaggtgaaccagtttggcggctacaccggtatgactcctgccgacttccgcgagatggtcttctccattgctgaagacattggccttcctaagaacaaaatcattctcggcggcgaccacctcggtcccaatccgtggaagggtcagccttccgaccaggctatgcggaacgctattgaaatgattcgcgagtacgccaaagcaggctttaccaaactccacttggacgcttcaatgcggctggctgacgatcctggaaacgagaacgagcccttgaacccagaagtcattgcagagcggactgctctcttgtgcctggaagccgaacgtgcctttaaagaatccgcaggttctctccgccctgtttacgtcattggcacggacgttccgccaccaggaggtgctcagaatgagggaaagagcattcacgttacctccgtgcaggacttcgaacgtaccgttgagcttaccaagaaagcattctttgaccatggtctctatgaggcctggggccgtgtgatcgccgttgttgtgcagcccggcgttgaattcggtaacgagcacatttttgaatatgatcggaaccgtgcacgcgaattgaccgaagctatcaaaaaacaccctaacattgttttcgaaggccatagcacggactaccagacggccaaagcattgaaggaaatggttgaagacggagtagcaattttgaaggtaggccccgcactgacctttgcgcttcgggaagcattttttgcgctttcttccatcgagaaggaacttttctacgatacccctggactttgtagcaacttcgttgaagttgtagagcgggctatgctggacaaccctaagcactgggaaaagtactaccagggagaggaacgggagaatcggcttgcacgcaaatacagctttcttgaccgcctccgttactattggaatctgcccgaggtacgtactgccgtgaataagttgatcaccaatttggaaacgaaagaaatcccattgacgctcattagccagttcatgccgatgcagtatcaaaagattcgcaatggtctgctgcggaaagatcccatctctctgatcaaggaccggatcaccttggtcctggacgattactattttgcaacccatcctgaatgt

SEQ ID NO: 4 - DNA, 1305 bp, Artificial Sequence
  Kosmotoga olearia fructose-4-epimerase Variant polynucleotide_WVY_ polynucleotide
atgaaaaagcatccattgcaggacatcgtatcactgcagaagcagggtatccccaagggcgtcttctcagtctgttccgctaaccgtttcgtcatcgagaccactctggaatacgccaagatgaagggcactacggttcttattgaagcaacctgtaaccaggtgaaccagtttggcggctacaccggtatgactcctgccgacttccgcgagatggtcttctccattgctgaagacattggccttcctaagaacaaaatcattctcggcggcgaccacctcggtccctacccgtggaagggtcagccttccgaccaggctatgcggaacgctattgaaatgattcgcgagtacgccaaagcaggcttttggaaactccacttggacgcttcaatgcggctggctgacgatcctggaaacgagaacgagcccttgaacccagaagtcattgcagagcggactgctctcttgtgcctggaagccgaacgtgcctttaaagaatccgcaggttctctccgccctgtttacgtcattggcacggacgttccgccaccaggaggtgctcagaatgagggaaagagcattcacgttacctccgtgcaggacttcgaacgtaccgttgagcttaccaagaaagcattctttgaccatggtctctatgaggcctggggccgtgtgatcgccgttgttgtgcagcccggcgttgaattcggtaacgagcacatttttgaatatgatcggaaccgtgcacgcgaattgaccgaagctatcaaaaaacaccctaacattgttttcgaaggccatagcacggactaccagacggccaaagcattgaaggaaatggttgaagacggagtagcaattttgaaggtaggccccgcactgacctttgcgcttcgggaagcattttttgcgctttcttccatcgagaaggaacttttctacgatacccctggactttgtagcaacttcgttgaagttgtagagcgggctatgctggacaaccctaagcactgggaaaagtactaccagggagaggaacgggagaatcggcttgcacgcaaatacagctttcttgaccgcctccgttactattgggttctgcccgaggtacgtactgccgtgaataagttgatcaccaatttggaaacgaaagaaatcccattgacgctcattagccagttcatgccgatgcagtatcaaaagattcgcaatggtctgctgcggaaagatcccatctctctgatcaaggaccggatcaccttggtcctggacgattactattttgcaacccatcctgaatgt

SEQ ID NO: 5 - protein, 435 aa, Artificial Sequence
  Kosmotoga olearia fructose-4-epimerase Variant_WVY_amino acid
MKKHPLQDIVSLQKQGIPKGVFSVCSANRFVIETTLEYAKMKGTTVLIEATCNQVNQFGGYTGMTPADFREMVFSIAEDIGLPKNKIILGGDHLGPYPWKGQPSDQAMRNAIEMIREYAKAGFWKLHLDASMRLADDPGNENEPLNPEVIAERTALLCLEAERAFKESAGSLRPVYVIGTDVPPPGGAQNEGKSIHVTSVQDFERTVELTKKAFFDHGLYEAWGRVIAVVVQPGVEFGNEHIFEYDRNRARELTEAIKKHPNIVFEGHSTDYQTAKALKEMVEDGVAILKVGPALTFALREAFFALSSIEKELFYDTPGLCSNFVEVVERAMLDNPKHWEKYYQGEERENRLARKYSFLDRLRYYWVLPEVRTAVNKLITNLETKEIPLTLISQFMPMQYQKIRNGLLRKDPISLIKDRITLVLDDYYFATHPEC

SEQ ID NO: 6 - DNA, 1308 bp, Artificial Sequence
  Kosmotoga olearia fructose-4-epimerase Variant polynucleotide_W_ polynucleotide
atgaaaaagcatccattgcaggacatcgtatcactgcagaagcagggtatccccaagggcgtcttctcagtctgttccgctaaccgtttcgtcatcgagaccactctggaatacgccaagatgaagggcactacggttcttattgaagcaacctgtaaccaggtgaaccagtttggcggctacaccggtatgactcctgccgacttccgcgagatggtcttctccattgctgaagacattggccttcctaagaacaaaatcattctcggcggcgaccacctcggtcccaatccgtggaagggtcagccttccgaccaggctatgcggaacgctattgaaatgattcgcgagtacgccaaagcaggcttttggaaactccacttggacgcttcaatgcggctggctgacgatcctggaaacgagaacgagcccttgaacccagaagtcattgcagagcggactgctctcttgtgcctggaagccgaacgtgcctttaaagaatccgcaggttctctccgccctgtttacgtcattggcacggacgttccgccaccaggaggtgctcagaatgagggaaagagcattcacgttacctccgtgcaggacttcgaacgtaccgttgagcttaccaagaaagcattctttgaccatggtctctatgaggcctggggccgtgtgatcgccgttgttgtgcagcccggcgttgaattcggtaacgagcacatttttgaatatgatcggaaccgtgcacgcgaattgaccgaagctatcaaaaaacaccctaacattgttttcgaaggccatagcacggactaccagacggccaaagcattgaaggaaatggttgaagacggagtagcaattttgaaggtaggccccgcactgacctttgcgcttcgggaagcattttttgcgctttcttccatcgagaaggaacttttctacgatacccctggactttgtagcaacttcgttgaagttgtagagcgggctatgctggacaaccctaagcactgggaaaagtactaccagggagaggaacgggagaatcggcttgcacgcaaatacagctttcttgaccgcctccgttactattggaatctgcccgaggtacgtactgccgtgaataagttgatcaccaatttggaaacgaaagaaatcccattgacgctcattagccagttcatgccgatgcagtatcaaaagattcgcaatggtctgctgcggaaagatcccatctctctgatcaaggaccggatcaccttggtcctggacgattactattttgcaacccatcctgaatgttga

SEQ ID NO: 7 - protein, 435 aa, Artificial Sequence
  Kosmotoga olearia fructose-4-epimerase Variant_W_amino acid
MKKHPLQDIVSLQKQGIPKGVFSVCSANRFVIETTLEYAKMKGTTVLIEATCNQVNQFGGYTGMTPADFREMVFSIAEDIGLPKNKIILGGDHLGPNPWKGQPSDQAMRNAIEMIREYAKAGFWKLHLDASMRLADDPGNENEPLNPEVIAERTALLCLEAERAFKESAGSLRPVYVIGTDVPPPGGAQNEGKSIHVTSVQDFERTVELTKKAFFDHGLYEAWGRVIAVVVQPGVEFGNEHIFEYDRNRARELTEAIKKHPNIVFEGHSTDYQTAKALKEMVEDGVAILKVGPALTFALREAFFALSSIEKELFYDTPGLCSNFVEVVERAMLDNPKHWEKYYQGEERENRLARKYSFLDRLRYYWNLPEVRTAVNKLITNLETKEIPLTLISQFMPMQYQKIRNGLLRKDPISLIKDRITLVLDDYYFATHPEC

SEQ ID NO: 8 - DNA, 98 bp, Artificial Sequence
  pHCP7
gctgcacgaatacctgaaaaacgttgaacgccccgtgagcggtaactcacagggcgtcggctaacccccagtccaaacctgggagaaagcgctcaaaa

SEQ ID NO: 9 - protein, 481 aa, Unknown
  Thermotoga neapolitana fructose-4-epimerase
MVLKVFKDHFGRGYEVKGEEGKILVVAGEKAPKGEEGKILVVAGEKAPEGLSFFKKQRVEGVSFFFCERNHENLEVLRKYFPDLKPVRAGLRASFGTGDRLGITTPAHVRALKDSGLFPIFAQQSVRENERTGRTWRDVLDDATWGVFQEGYSEGFGADADHVKRPEDLVSAAREGFTMFTIDPSDHVRNLSKLSEREKNEMFEEILKKERIDRIYLGKKYTVLGERLEFDEKNLRDAALVYYDAIAHVDMMYQILKDETPDFDFEVSVDETETPTSPLFHIFVVEELRRRGVEFTNLALRFIGEWEKGIDYKGDLAQFEREIKMHAEIARMFEGYKISLHSGSDKFSVYPAFASATGGLFHVKTAGTSYLEAVKVISMVNPELFREIYRCALDHFEEDRKSYHISADLSKVPEVEKVKDEDLPGLFEDINVRQLIHVTYGSVLKDASLKERLFKTLEQNEELFYETVAKHIKRHVDLLKG

SEQ ID NO: 10 - protein, 481 aa, Artificial Sequence
  Thermotoga neapolitana fructose-4-epimerase Variant
MVLKVFKDHFGRGYEVKGEEGKILVVAGEKAPKGEEGKILVVAGEKAPEGLSFFKKQRVEGVSFFFCERNHENLEVLRKYFPDLKPVRAGLRASFGTGDRLGITTPAHVRALKDSGLFPIFAQQDVRENERTGRTWRDVLDDATWGVFQEGYSEGFGADADHVKRPEDLVSAAREGFTMFTIDPQDHVRNLSKLSEREKNEMFEEILKKERIDRIYLGKKYTVLGERLEFDEKNLRDAALVYYDAIAHVDMMYQILKDETPDFDFEMTVDEDETPTSPLFHIFVVEELRRRGVEFTNLALRFIGEMEKGIDYKGDLAQFEREIKMHAEIARMFEGYKISLHSGSDKFSVYPAFASATGGLFHVKTAGTSYLEAVKVISMVNPELFVEIYRCALDHFEEDRKSTHISADLSKVPEVEKVKDEDLPGLFEDINVRQLIHVTYGSVLKDASLKERLFKTLEQNEELFYETVAKHIKRHVDLLKG

SEQ ID NO: 11 - DNA, 1447 bp, Artificial Sequence
  Thermotoga neapolitana fructose-4-epimerase_ polynucleotide
atggtcttgaaagtgttcaaagatcactttggaaggggatacgaagtttacgaaaagtcttatagagaaaaggattctctctctttcttcttgacaaagggagaggaaggaaaaattctggtagtggctggagaaaaggcacctgagggtctgtcgtttttcaaaaaacagcgggtggagggtgtttcgttctttttctgtgagagaaatcatgagaacttggaagttctcagaaaatactttccagatctcaaaccagttcgagcgggattgagagcgtcttttggaacaggtgacagactcggtatcaccacaccggctcacgtgagggcgttgaaggattcagggctttttcccatctttgcgcagcaggacgtgagggagaacgagagaacgggaaggacctggagagatgtgctggacgatgccacatggggagttttccaggagggatacagtgagggattcggagcagacgccgatcacgtgaagcggccggaggatcttgtttcggctgcaagggaaggtttcaccatgttcacaatcgatcctcaggatcatgtgaggaatctttcaaaactcagtgaaagagaaaagaacgagatgttcgaggaaatactgaaaaaagagcgaatcgacaggatctatcttgggaaaaaatacaccgtcctcggtgaaagactggagttcgacgagaaaaatttgagggatgctgctctggtgtactatgatgcgatcgcccacgtggatatgatgtatcaaattttgaaagacgaaaccccggatttcgacttcgaaatgacagttgacgaagatgaaactcccacgagtcctctcttccacattttcgttgtggaagaactcagacgaagaggtgtggagttcaccaatcttgccctgagattcatcggcgaaatggaaaagggaatagattacaagggggatcttgcacagttcgagagagaaatcaaaatgcacgcagaaatcgcaaggatgttcgaaggatacaaaatatcactccactctggaagcgacaaattttccgtgtatcctgcttttgcttccgcgacaggaggccttttccacgtgaagacagccggaacgagttatcttgaggcggtgaaggtcatatccatggtcaacccggagctcttcgttgagatctacaggtgtgctctcgatcactttgaggaagacagaaagtccacacacatatctgcggatctgtcgaaagttccggaagtagagaaagtgaaagatgaagatcttccaggtctttttgaagacatcaacgtgagacagttgatccatgtcacctatggctctgttctgaaagatgcatctttgaaagaacggctgtttaagacgcttgaacaaaatgaggaactcttctacgagaccgtggcaaaacatataaaaaggcacgtagacctgttgaaggggctaa

SEQ ID NO: 12 - DNA, 1446 bp, Artificial Sequence
  variant 2
atggtcctgaaagtcttcaaggaccactttggacgaggatacgaagtttacgaaaagtcttaccgcgaaaaggactctctttctttcttcctgaccaagggagaggaaggcaaaatcctcgttgtggccggtgaaaaagcacctgagggcctgtcgtttttcaagaaacagcgagtggagggagtctcgttctttttctgtgagcgcaatcatgagaacctcgaagtactgcgtaaatactttccagaccttaagccagtgcgcgcaggtcttcgtgcctcttttggaaccggcgaccgccttggcatcaccaccccggcacacgttcgcgcacttaaggactcaggtctctttcccatctttgctcagcaggacgtccgcgagaacgagcgcaccggacgcacctggcgagacgttcttgacgatgctacctggggtgtgttccaggagggctactccgagggcttcggtgcagacgctgatcacgttaagcgcccggaggacctcgtatcggctgcacgtgaaggattcaccatgttcactatcgatcctcaggaccacgttcgcaatctctcaaaactgtccgaacgcgaaaagaacgagatgttcgaggaaattcttaaaaaggagcgcatcgatcgtatctacttgggaaaaaaatataccgtccttggagaacgcctggagttcgacgagaaaaatctgcgcgacgctgcacttgtctactatgacgccatcgcacacgttgacatgatgtaccaaatcttgaaagatgaaactccggacttcgacttcgaaatgaccgtcgatgaagatgaaactcccacttcccctctgttccacatcttcgtcgtggaagaactgcgccgccgtggcgttgagttcacgaatctggcactccgcttcatcggcgaaatggaaaaaggcatcgactacaaaggtgacctggcccagttcgagcgcgaaatcaaaatgcacgctgaaatcgcacgcatgttcgaaggatacaaaatttcactccactctggaagcgacaaattttccgtctaccctgcatttgcttccgccacgggaggactcttccacgtgaaaaccgcaggtacgtcctacctggaggcagtcaaagtcatctccatggtgaacccggagctgttcgttgagatctatcgctgcgcactggaccattttgaggaagaccgtaagtccactcacatctctgcagatctgtcgaaggtgccggaagtcgagaaggtcaaagacgaagaccttccaggtctttttgaagacatcaacgttcgccagttgatccacgtcacctacggctctgtcctgaaagatgcttctttgaaggaacgcctctttaaaaccctcgaacaaaatgaggaactcttctacgagaccgttgctaaacacatcaagcgccacgttgatctcttgaaaggataa

SEQ ID NO: 13 - DNA, 1446 bp, Artificial Sequence
  variant 1
atggtgctgaaggtgttcaaggatcacttcggccgcggctacgaagtgtacgaaaagtcctaccgcgaaaaggactccctgtccttcttcctgaccaagggcgaagaaggcaagatcctggtggtggccggcgaaaaggccccagaaggcctgtccttctttaagaagcagcgcgtggaaggcgtgtccttcttcttctgcgaacgcaaccacgaaaacctggaagtgctgcgcaagtacttcccagatctgaagccagtgcgcgccggcctgcgcgcatctttcggtactggcgaccgcctgggcatcaccaccccagctcacgtgcgcgccctgaaggactccggcctgttcccaatcttcgcccagcaggacgtgcgcgaaaacgaacgcaccggccgcacctggcgcgacgttttggacgacgcaacctggggcgtgttccaggaaggctactccgaaggcttcggcgcagatgcagatcacgtgaagcgcccagaagatctggtgtccgcagcacgcgaaggcttcaccatgttcaccatcgacccacaggatcacgtgcgcaacctgtccaagctgtccgaacgcgaaaagaacgaaatgttcgaagaaatcctgaagaaggaacgcatcgaccgcatctacctgggcaagaagtacaccgtgctgggcgaacgcctggaattcgatgaaaagaacctgcgcgatgccgcactggtgtactacgatgccatcgcccacgtggacatgatgtaccagatcctgaaggatgaaaccccagacttcgacttcgaaatgaccgtggatgaagacgaaaccccaacctccccactgttccacatcttcgtggtggaagaactgcgccgccgcggcgtggaattcaccaacctggcactgcgcttcatcggcgaaatggaaaagggcatcgactacaagggcgacctggcacagttcgaacgcgaaatcaagatgcacgcagaaatcgcacgcatgttcgaaggctacaagatctccctgcactccggctccgataagttctccgtgtacccagcattcgcatccgcaaccggcggcctgttccacgtgaagaccgcaggcacctcctacctggaagccgtgaaggtcatttccatggtgaacccagaactgttcgtggaaatctaccgctgcgcactggatcacttcgaagaagatcgcaagtccacccacatctccgccgatctgtccaaggtgccagaagtggaaaaggtgaaggatgaagacctgccaggcctgttcgaagacatcaacgtgcgccagctgatccacgtgacctacggctccgtgctgaaggacgcctccctgaaggaacgcctgttcaagaccctggaacagaacgaagaactgttctacgaaaccgtggccaagcacatcaagcgccacgtggacctgctgaagggctaa